European Patent Application EP 4 810 526 A1, published September 23, 2026. Title: 具有靶向功能的分子及应用. Applicant: 深圳虹信生物科技有限公司. Application CN 2023116272306, filed November 30, 2023. The sequence listing filed with the application follows.

SEQUENCE LISTING (85 sequences)

SEQ ID NO: 1 - protein, 132 aa, synthetic construct
QVQLQESGGGSVQPGGSLRLSCAASGFTFDDYAMSWVRQVPGKGLEWVSTINWNGGSAEYAEPVKGRFTISRDNAKNTVYLQMNSLKLEDTAVYYCAKDADLVWYNLSTGQGTQVTVSSAAAYPYDVPDYGS

SEQ ID NO: 2 - protein, 132 aa, synthetic construct
QVQLQESGGGLVQPGGSLRLSCAASGFTFDDYAMSWVRQVPGKGLEWVSTINWNGGSAEYAEPVKGRFTISRDNAKNTVYLQMNSLKLEDTAVYYCAKDADLVWYNLRTGQGTQVTVSSAAAYPYDVPDYGS

SEQ ID NO: 3 - protein, 144 aa, synthetic construct
QVQLQESGGGLVQAGGSLRLSCAASGFTFDDYAIGWFRQAPGKEREGVSCIRVSDGSTYYADPVKGRFTISSDNAKNTVYLQMNSLKPEDAAVYYCAAGSLYTCVQSIVVPARPYYDMDYWGKGTQVTVSSAAAYPYDVPDYGS

SEQ ID NO: 4 - protein, 124 aa, synthetic construct
DVQLQESGGGLVQPGDSLRLSCAASGRTFSSYDMGWFRQAPGKEREFVAAISRSGRDTLHADSVKGRFTISRDNAKNTVYLQMNSLKPEDTAVYICAGTGFEYAGSTPYKYPYWGQGTQVTVSS

SEQ ID NO: 5 - protein, 119 aa, synthetic construct
DVQLQESGGGLVQAGGSLRLSCTASGSIVSIISMGWYRQAPGKQRELIAKITTDGTTNYADSVRGRFTISRDIPKKIMYLQMSSLTPEDTAVYFCNRDRLLYGLVKSDWGQGTQVTVSS

SEQ ID NO: 6 - protein, 123 aa, synthetic construct
DVQLQESGGGFVRPGGSLRLSCAASGPTVSSYTVGWFRQAPGKEREYVATISWSDASTYYADFVKGRFTISRDYAKQVVYLQMNSLKPEDTAVYHCAAVFRRVPISATLYDYWGQGTQVTVSS

SEQ ID NO: 7 - protein, 112 aa, synthetic construct
DVQLQESGGGLVQPGGSLRLSCAASGSAFSRIGVGWYRQAPGKEREFVAVITAGGNTNYADSVKGRFTISRDNAKNTVYLQMNSLKPEDTGVYYCNYPGRPWGQGTQVTVSS

SEQ ID NO: 8 - protein, 112 aa, synthetic construct
DVQLQESGGGLVQPGGSLRLSCAASGSAFSRIGVGWYRQAPGKEREFVAVITAGGNTNYADSVKGRFTISRDNAKNTVYLQMNSLKPGDTGVYYCNYPGRPWGQGTQVTVSS

SEQ ID NO: 9 - protein, 121 aa, synthetic construct
DVQLQESGGGLVQPGGSLRLACAASGNIFEIHAMYWYRQAPGKQREWVAAITTRGSTNVADSVKGRFTISRDNAKNTVYLQMNSLKPEDTAVYLCNADVFSALTGAGTEYWGQGTQVTVSS

SEQ ID NO: 10 - protein, 112 aa, synthetic construct
DVQLQESGGGLVQPGGSLRLSCVASGSAFSRIGVGWYRQAPGKEREFVAEITAGGNTDYADSVKGRFTISRDNAKNMVYLQMNSLKPEDTGVYYCNYPGRPWGQGTQVTVSS

SEQ ID NO: 11 - protein, 126 aa, synthetic construct
DVQLQESGGGLVQAGGSLRLSCAASGHTLSIYAMTWFRQDSGKDREFVAAITWPDYSTYYADSVKGRFTISGDRPKNTVYLEMNSVKPEDTAVYYCAADRYVNSVPTATPQEWRYWGQGTQVTVSS

SEQ ID NO: 12 - protein, 126 aa, synthetic construct
DVQLQESGGGLVQAGGSLRLSCAVSGRTISGMSVGWFRQAPGKEREFVAADNWAGAKTSYADSVKGRFTISRDNAKAMVYLQMNGLKPEDTAVYYCAGRTSDGLSTYARIEDYYGWGQGTQVTVSS

SEQ ID NO: 13 - protein, 115 aa, synthetic construct
DVQLQESGGGLAQAGGSLRLSCAASGGIFSIDAAAWYRQAPGKERELVAHIFHGGSTTYEDSVKGRFTISRDNAKNTVYLQMNSLKPEDTAVYYCYGGPPGMAIWGKGTQVTVSS

SEQ ID NO: 14 - protein, 130 aa, synthetic construct
DVQLQESGGGLVQAGASLSLSCAASGRTVNYVFGMGWFRQALGKEREFVAAITRSGGIPLYADSVKGRFTISRDNAKNTVYLQMNSLKPEDTAVYYCAIDRQYYSGRNYPQSDPAEYDYWGQGTQVTVSS

SEQ ID NO: 15 - protein, 125 aa, synthetic construct
DVQLQESGGGLVQAGGSLRLSCAASVRTFSKYDIGWFRQAPGKEREFVATISSSGRSTYYADFAKGRFGISRDYAKNTVYLEMNSLKPEDTAVYACAVRLGYSGSETDPRQYAYWGQGTQVTVSS

SEQ ID NO: 16 - protein, 123 aa, synthetic construct
DVQLQESGGGFVQPGGSLRLSCAASGPTVSSYTVGWFRQAPGKEREYVATISWSDASTYYADFVKGRFTISRDYAKQVVYLQMNSLKPEDTAVYHCAAVFRRVPISATLYDYWGQGTQVTVSS

SEQ ID NO: 17 - protein, 115 aa, synthetic construct
DVQLQESGGGLVQAGDSLRLSCAPSGGIFSINAAAWYRQAPGKERELVAHINHGGSTTYVGSVKGRFTISRDNAKNTVYLQMNSLKPEDTAVYYCYGGPPGMAIWGKGTQVTVSS

SEQ ID NO: 18 - protein, 110 aa, synthetic construct
DVQLQESGGGLVQAGGSLRLSCTASGTIFNVMGWYRQAPGKQRELVATITFGLTTNYADSVKGRFAISRDNSEKTVYLQMNSLKPEDTAVYYCNAGSRYWGQGTQVTVSS

SEQ ID NO: 19 - protein, 126 aa, synthetic construct
DVQLQESGGGLVQAGGSLRLSCAASGRTFSSYAMGWFRQAPGKEREFVAAISWSGGSTTEADSVKGRFTISRDNAKNTVYLQMYSLKPEDTAVYYCAAARDLVSTVVAETSEYDYWGQGTQVTVSS

SEQ ID NO: 20 - protein, 126 aa, synthetic construct
DVQLQESGGGLVQAGGSLRLSCAVSGRTINDMSVGWFRQAPGKEREFVAADIWPGAKTSYADPVKGRFTITRDNAKAMVYLQMNGLKPEDTAVYYCAGRTSDGLRTYTRIEDYYGWGQGTQVTVSS

SEQ ID NO: 21 - protein, 116 aa, synthetic construct
DVQLQESGGGLVQPGGSLRLACAASGSGFSINAMGWYRQAPGKQREWVAAINSVGMTNYRDSVKGRFTISRDDAKNTVYLQMNSLKPEDTAVYYCNVKPLGTADYWGQGTQVTVSS

SEQ ID NO: 22 - protein, 126 aa, synthetic construct
DVQLQESGGGLVQAGGSLRLSCAVSGRTISGMSVGWFRQAPGKEREFVAADSWAGAKTSYADSVKGRFTISRDNAKAMVYLQMKGLKPEDTAVYYCAGRTSDGLFNYARIEDYYGWGQGTQVTVSS

SEQ ID NO: 23 - protein, 126 aa, synthetic construct
DVQLQESGGGLVQAGDSLRLSCAVSGRTISGMSVGWFRQAPGKEREFVAADSSAGAKTSYADSVKGRFTISRDNAKAMVYLQMNGLKPEDTAVYYCAGRTSYGLSTYARMEDYYGWGQGTQVTVSS

SEQ ID NO: 24 - protein, 123 aa, synthetic construct
DVQLQESGGGLVQPGGSLRLSCAASGSIFSSNVMGWYRQAPGKQREWVSTIISDGRTNYAGSVKGRFTISRDNAKNTVYLQMNNLKPEDTALYYCKLSTLNRDYWGQGTLVTVGQGTQVTVSS

SEQ ID NO: 25 - protein, 125 aa, synthetic construct
DVQLQESGGGLVQAGGSLRLSCAASGRTSTIYTMGWFRQAPGKEREFVAATSWSGGNTNYAASMKGRFTISRNNAKNTVYLQMNSLKPEDTAVYYCAANRGSYYLGPSPYEYDWWGQGTQVTVSS

SEQ ID NO: 26 - protein, 120 aa, synthetic construct
DVQLQESGGGLVQPGGSLRLSCAASGSIFSINAMGWYRQAPGKQRDVVAYIMSDGNTHYADSVKGRFTISRDENTSYLQMNSLKPDDTAVYYCNADIQPPMPEATIYVYWGQGTQVTVSS

SEQ ID NO: 27 - protein, 119 aa, synthetic construct
DVQLQESGGGLVQTGGSLRVSCAASGRTFSSAYMGWFRQAPGKERVLVAEIWLSSGQTYYADSVKGRFTISRENAKNTVYLQMNSLKPEDTAVYYCAAQNRATGRYDYWGQGTQVTVSS

SEQ ID NO: 28 - protein, 123 aa, synthetic construct
DVQLQESGGGLVQPGGSLRLSCAASGSIFSSNVMGWYRQAPGKQREWVSTIISDGRTNYAGSVKGRFTISRDNAKNTVYLQMNNLKPEDTALYYCKLSTLNRDYWGQGTQVTVGQGTQVTVSS

SEQ ID NO: 29 - protein, 115 aa, synthetic construct
DVQLQESGGGLVQPGGSLRLSCAASGGIFSINAAAWYRQAPGKERELVAHIYHGGSTTYVGSVKGRFTISRDNAKNTVYLQMNSLKPEDTAVYYCYGGPPGMAIWGKGTQVTVSS

SEQ ID NO: 30 - protein, 123 aa, synthetic construct
DVQLQESGGGFVQPGGSLRLSCAASGPTVSSYTVGWFRQAPGKEREYVATISWSDASTYYADFVKGRFTISRDYAKKVVYLQMNSLKPEDTAVYHCAAVFRRVPISATLYDYWGQGTQVTVSS

SEQ ID NO: 31 - protein, 115 aa, synthetic construct
DVQLQESGGGLVQAGGSLRLSCAASGGIFSINAAAWYRQAPGKERELVAHITHGGSTTYEGSVKGRFTISKDNAKNTVYLQMNSLKPEDTAVYYCYGGPPGMAIWGKGTQVTVSS

SEQ ID NO: 32 - protein, 119 aa, synthetic construct
DVQLQESGGGLVQAGGSLRLSCAASGSIVSIISVGWYRQAPGKQRELVAKITTDGTTNYADSVRGRFTISRDIAKKMLYLQMSSLTPEDTAVYFCNRDRLVYGLVKADWGQGTQVTVSS

SEQ ID NO: 33 - protein, 125 aa, synthetic construct
DVQLQESGGGLVQAGGSLRLSCAASGRTSTIYTMGWFRQAPGREREFVAATSWSGGNTNYAGSVKGRFTISRNDAKNTVYLQMNSLKPEDTAVYYCAANRGSYYLGPSFYEYDYWGQGTQVTVSS

SEQ ID NO: 34 - protein, 119 aa, synthetic construct
DVQLQESGGGLVQAGGSLRLSCTASGSIVSIISMGWYRQAPGKQRELIAKITTDGTTNYADSVRGRFTTSRDIPKKIMYLQMSSLTPEDTAVYFCNRDRLLYGLVKSDWGQGTQVTVSS

SEQ ID NO: 35 - protein, 119 aa, synthetic construct
DVQLQESGGGLVQTGGSLRVSCAASGRTFSSSYMGWFRQAPGQERELVAEIWLSSGQTYYADSVKGRFTISRENAKNTAYLQMNSLTPEDTAVYYCAAQNRATGRYDYWGQGTQVTVSS

SEQ ID NO: 36 - protein, 119 aa, synthetic construct
DVQLQESGGGLVQAGGSLRLSCTASGSIVSIISMGWYRQAPGKQRELIAKITTDGTTSYADSVRGRFTISRDIPKKIMYLQMSSLTPEDTAVYFCNRDRLLYGLVKSDWGQGTQVTVSS

SEQ ID NO: 37 - protein, 115 aa, synthetic construct
DVQLQESGGGLVQAGGSLRLSCAASGGIFSINAAAWYRQAPGKERELVAHIYHGGSTTYVGSVKGRFTISRDNAKNTVYLQMNSLKPEDTAVYYCYGGPPGMAIWGKGTQVTVSS

SEQ ID NO: 38 - protein, 128 aa, synthetic construct
DVQLQESGGGLVQAGGSLRLSCAASGRTFSSTGMGWFRQAPGKEREFVAAINWSGEDTYYADSVKGRFTISGDNAKNVVYLQMNSLKPEDTAVYYCAASPYYNPYGPRLRTPSWYDYWGQGTQVTVSS

SEQ ID NO: 39 - protein, 128 aa, synthetic construct
DVQLQESGGGLVQAGGSLRLSCAASGGTFSSSGMGWYRQAPGKEREFVAAINWSGEDTLYADSVKGRFTISGDNAKNTVHLQMNSLKPEDTAVYYCAASPYYNPYGPRLRTPSWYDYWGQGTQVTVSS

SEQ ID NO: 40 - protein, 110 aa, synthetic construct
DVQLQESGGGLVQAGGSLRLSCTASGTIFNVMGWYRQAPGKQRELVATITFDLSTNYADSVKGRFAISRDVTEKTVYLQMDSLKPEDTAVYYCNAGSRYWGQGTQVTVSS

SEQ ID NO: 41 - protein, 116 aa, synthetic construct
DVQLQESGGGLVQAGGSLRLSCAASGSTSGYSFRFWTMNWYRQGSGKQRELVATITSSGITTYADSVKGRFTVSRDNTKNTLYLQMNSLKPEDTATYYCNFPGNSWGQGTQVTVSS

SEQ ID NO: 42 - protein, 126 aa, synthetic construct
DVQLQESGGGLVQAGDSLRLSCAVSGRTISDMSVGWFRQAPGKEREFVAADSWAGAKTSYADSVKGRFTISRNNAKAMVYLQMNGLKPEDTAVYYCAGRTSDGLSTYEWIEDYYGWGQGTQVTVSS

SEQ ID NO: 43 - protein, 115 aa, synthetic construct
DVQLQESGGGLVQAGDSLRLSCVASGGIFSINAAAWYRQAPGKERELVAHIYHGGSTTYVGSVKGRFTISRDNAKNTVYLQMNSLKPEDTAVYYCYGGPPGMAIWGKGTQVTVSS

SEQ ID NO: 44 - protein, 114 aa, synthetic construct
DVQLQESGGGLVQPGGSLTLSCAASGSIFSRDVMGWYRQAPGKQRELVAAITIGGYADYADSVKGRFTISRDNAKNTVYLRMNSLKPEDTAVYFCKLGYGSGSWGQGTQVTVSS

SEQ ID NO: 45 - protein, 120 aa, synthetic construct
DVQLQESGGGLVQPGGSLRLSCAASRSTFSIDIMAWYRQAPEKKRELVALITRRGTTNYADSVKGRFTISRDNAKNTMYLQMNNLKPEDTAVYYCNSDDTETRWGLRQYWGQGTQVTVSS

SEQ ID NO: 46 - protein, 126 aa, synthetic construct
DVQLQESGGGLVQAGGSLRLSCAASGHTLSIYAMTWFRQDSGKDREFVAAITWPDYSTYYADSVKGRFTISGDRPKNTVHLEMNSVKPEDTAVYYCAADRYVNSVPTATPQEWRYWGQGTQVTVSS

SEQ ID NO: 47 - protein, 130 aa, synthetic construct
DVQLQESGGGLVQPGASLSLSCAASGRTVNYVFGMGWFRQALGKEREFVAAITRSGGIPLYADSVKGRFTISRDNAKNTVYLQMNSLKPEDTAVYYCAIDRQYYSGRNYPQSDPAEYDYWGQGTQVTVSS

SEQ ID NO: 48 - protein, 119 aa, synthetic construct
DVQLQESGGGLVQAGGSLRLSCSASGSIVSIISMGWYRQAPGKQRELIAKITTDGTTNYADSVRGRFTISRDIPKKIMYLQMSSLTPEDTAVYFCNRDRLLYGLVKSDWGQGTQVTVSS

SEQ ID NO: 49 - protein, 115 aa, synthetic construct
DVQLQESGGGLVQAGGSLRLSCAASGGIFSINAAAWYRQAPGKERELVAHIFHGGSTTYEDSVKGRFTISRDNAKNTVYLQMNSLKPEDTAVYYCYGGPPGMAIWGKGTQVTVSS

SEQ ID NO: 50 - protein, 120 aa, synthetic construct
DVQLQESGGGLVQPGGSLRLSCAASGSIFSINAMGWYRQAPGKQRDVVAYIMSDGNTHYADSVKGRFTISRDKNTSYLQMNSLKPDDTAVYYCNADIQPPMPEATIYVYWGQGTQVTVSS

SEQ ID NO: 51 - protein, 110 aa, synthetic construct
DVQLQESGGGLVQAGGSLRLSCTASGTIFNVMGWYRQAPGKQRELVATITFGLATNYADSVKGRFAISRDDSEKTVYLQMNSLKPEDTAVYYCNAGSRYWGQGTQVTVSS

SEQ ID NO: 52 - protein, 116 aa, synthetic construct
DVQLQESGGGLVQAGGSLRLSCAASGSTSGYSFGFWTMNWYRQGSGKQRELVATITSSGITTYADSVKGRFTVSRDNTKNTLYLQMNSLKPEDTATYYCNFPGNSWGQGTQVTVSS

SEQ ID NO: 53 - protein, 119 aa, synthetic construct
DVQLQESGGGLVQAGGSLRLSCTASGSIVSIISMGWYRQAPGKQRELIAKVTTDGTTNYADSVRGRFTISRDIPKKIMYLQMSSLTPEDTAVYFCNRDRLLYGLVKSDWGQGTQVTVSS

SEQ ID NO: 54 - protein, 121 aa, synthetic construct
DVQLQESGGGLVQPGGSLRLSCLVSGSIYSIPAMYWYRQAPGKQREFVADITNRGSTNYADSVKGRFTISRDNAKNTVNLQMNSLKPEDTAVYYCNVLGTLGPRGSLQDYWGQGTQVTVSS

SEQ ID NO: 55 - protein, 119 aa, synthetic construct
DVQLQESGGGLVQPGGSLRLSCTASGSIVSIISMGWYRQAPGKQRELIAKITTDGTTNYADSVRGRFTISRDIPKKIMYLQMSSLTPEDTAVYFCNRDRLLYGLVKSDWGQGTQVTVSS

SEQ ID NO: 56 - protein, 125 aa, synthetic construct
DVQLQESGGGLVQAGGSLRLSCAASVRTFSKYDIGWFRQAPGKEREFVATISSSGRSTYYADFVKGRFGISRDYAKNTVYLEMNSLKPEDTAVYACAVRLGYSGSETDPRQYAYWGQGTQVTVSS

SEQ ID NO: 57 - protein, 119 aa, synthetic construct
DVQLQESGGGLVQAGGSLRLSCTASGSIVSIISMGWYRQAPGKQRELIAKITTDGTTNYADSVRGRFTISRGIPKKIMYLQMSSLTPEDTAVYFCNRDRLLYGLVKSDWGQGTQVTVSS

SEQ ID NO: 58 - protein, 129 aa, synthetic construct
DVQLQESGGGLVQTGGSLRLSCAASGRTFEHYTMGMGWFRQAPGKEREFVAAISWSDGSTYYEDSVKGRFTISRGNAKTTVYLQMNSLEPEDTGVYICAAKRGIGSDYPATLLYEYDYWGQGTQVTVSS

SEQ ID NO: 59 - protein, 126 aa, synthetic construct
DVQLQESGGGLVQAGGSLRLSCAVSGRTISDMSVGWFRQAPGKEREFVAADTWAGAKTSYADSVKGRFTISRDTAKAMVYLQMNGLKPEDTAVYYCAGRTSYGLSTYARIEDYYGWGQGTQVTVSS

SEQ ID NO: 60 - protein, 123 aa, synthetic construct
DVQLQESGGGLVQAGGSLRLSCAASGRTFNTNAMGWFRQAPGKEREFVAAIDWSGDSTFYADSVKGRFTISRDNAKNTVYLQMNSLKPEDTAVYYCAADGLLYYSGSYYPDYWGQGTQVTVSS

SEQ ID NO: 61 - protein, 126 aa, synthetic construct
DVQLQESGGGLVQAGGSLRLSCAVSGRTISDMSVGWFRQAPGKEREFVAADSWAGAKASYADSVKGRFTISRDNTKAMVHLQMNGLKPEDTAVYYCAGRTSDGLSTYARIEDYYGWGQGTQVTVSS

SEQ ID NO: 62 - protein, 110 aa, synthetic construct
DVQLQESGGGLVQAGGSLRLSCTASGTIFNVMGWYRQAPGKQRELVATITFGLTTNYADSVKGRFAISRDSSEKTVYLQMNSLKPEDTAVYYCNAGSRYWGQGTQVTVSS

SEQ ID NO: 63 - protein, 126 aa, synthetic construct
DVQLQESGGGLVQAGGSLRLSCAVSGRTISDMSVGWFRQAPGKEREFVAADTWAGAKTSYADSVKGRFTISRDNAKAMVYLQMNGLKPEDTAVYYCAGRTSYGLSTYARIEDYYGWGQGTQVTVSS

SEQ ID NO: 64 - protein, 112 aa, synthetic construct
DVQLQESGGGLVQPGGSLRLSCAASGSAFSRIGVGWYRQAPGKEREFVAVITAGGNTNCADSVKGRFTISRDNAKNTVYLQMNSLKPEDTGVYYCNYPGRPWGQGTQVTVSS

SEQ ID NO: 65 - protein, 112 aa, synthetic construct
DVQLQESGGGLGQAGGSLRLSCAVSEIIFRFTTLNWYRQAPGKQRELVASISSGGSTNYDDSVKGRFTISRDNAKKLVYLQMNSLKPEDTAVYYCNVPGNPWGQGTQVTVSS

SEQ ID NO: 66 - protein, 126 aa, synthetic construct
DVQLQESGGGLVQPGGSLKLSCAVSGRTISGMSVGWFRQAPGKEREFVAADSWAGAKTSYADSVKGRFTISRDNAKAMVYLQMKGLKPEDTAVYYCAGRTSDGLFNYARIEDYYGWGQGTQVTVSS

SEQ ID NO: 67 - protein, 123 aa, synthetic construct
DVQLQESGGGFVQAGDSLRLSCAASGRAVISYTLGWFRQAPGKEREFVATISWTDGSTYYSDSVKGRFTMSRDDAKKTVYLQMNSLKPEDTAVYYCAAVFRRVPTSATLYDYWGQGTQVTVSS

SEQ ID NO: 68 - protein, 126 aa, synthetic construct
DVQLQESGGGLVQAGDSLRLSCAVSGRTISGMAVGWFRQAPGKEREFVAADSRAGAKTSYADSVKGRFTLSRDNAKAMVYLQMNGLKPEDTAVYYCAGRTSDGLSTYARIQDYYGWGQGTQVTVSS

SEQ ID NO: 69 - protein, 112 aa, synthetic construct
DVQLQESGGGLVQPGGSLRLSCAASGSAFSRIGVGWYRQAPGKEHEFVAEINAGGNTNYADSVKGRFTISRDNAKNTVYLQMNSLKPEDTGVYYCNYPGRPWGQGTQVTVSS

SEQ ID NO: 70 - protein, 122 aa, synthetic construct
DVQLQESGGGLVQPGGSLRLSCAASGRFFSISAMGWYRQAPGKQRELVAAIINGGGTHYADSVKGRFTISRDNAKNTVYLQMNSLKPEDTAVYYCNADAQMESGTLYFIVFWGQGTQVTVSS

SEQ ID NO: 71 - protein, 126 aa, synthetic construct
DVQLQESGGGLVQAGDSLRLSCAVSGRTISDMSVGWFRQAPGKEREFVAADSWAGAKTSYADSVKGRFTISRDNAKAMVYLQMNGLKPEDTAVYYCAGRTSDGLSTYARIEDYYGWGQGTQVTVSS

SEQ ID NO: 72 - protein, 124 aa, synthetic construct
DVQLQESGGGLVQPGDSLRLSCAASGRTFSSYDMGWFRQAPGKEREFVAAISRSGRDTLHADSVKGRFTISRDNAKNTVYLQMYSLKPEDTAVYICAGTGFEYAGSTPYKYPYWGQGTQVTVSS

SEQ ID NO: 73 - protein, 112 aa, synthetic construct
DVQLQESGGGLVQPGGSLRLSCAASGSAFSRIGVGWYRQAPGKEREFVAVIAAGGNTNYADSVKGRFTISRDNAKNTVYLQMNSLKPEDTGVYYCNYPGRPWGQGTQVTVSS

SEQ ID NO: 74 - protein, 114 aa, synthetic construct
DVQLQESGGGLVQAGGSLRLSCAASGGIFSRDVMGWYRQAPGEQRELVAAITIGGSASYADSVKGRFTISRDNAKNTVYLRMNSLTPEDTAVYFCKLGYGSGSWGQGTQVTVSS

SEQ ID NO: 75 - protein, 126 aa, synthetic construct
DVQLQESGGGLVQAGGSLRLSCVVSGRTLSGMSVGWFRQAPGKEREFVAADSWAGAKASYADSVKGRFTISRDNAEAIVYLQMNGLKPEDTAVYYCAGRTSYGLSTYARIEDYYGWGQGTQVTVSS

SEQ ID NO: 76 - protein, 126 aa, synthetic construct
DVQLQESGGGLVQAGGSLRLSCAVSGRTISGMSVGWFRQAPGKEREFVAADTWAGAKTSYADSVKGRFTISRDNTKAMVYLQMNGLKPEDTAVYYCAGRTSDGLSTYARIEDYYGWGQGTQVTVSS

SEQ ID NO: 77 - protein, 122 aa, synthetic construct
DVQLQESGGGLVQPGGSLRLSCAASGSIFSINAMGWYRQAPGKQRELVAHITNIGTTNYADSVKGRFTISRDNGKNTVYLQMNSLKPEDTAVYICNADLPSMVETDYYLVYWGQGTQVTVSS

SEQ ID NO: 78 - protein, 126 aa, synthetic construct
DVQLQESGGGLVQAGDSLRLSCAVSGRTISDMSVGWFRQAPGKEREFVAADSWAGAKTSYADSVKGRFTISRDNAKAMVYLQMSGLKPEDTAVYYCAGRTSSGLSTYARIEDYYGWGQGTQVTVSS

SEQ ID NO: 79 - protein, 123 aa, synthetic construct
QVQLQESGGGSVQAGGSLRLSCAAVSGITFRRNCMGWFRQVPGKEREGVATLDGASLTRYADSVKGRFIISQDNAKNTLYLQMNALKPEDTAMYYCAASPTRYGCGGADFDSWGQGTQVTVSS

SEQ ID NO: 80 - protein, 131 aa, synthetic construct
QVQLVESGGGLVQAGDSVTLSCTASGRTFSSYALAWFRQRPGKEREFVAGLRWGGPTNYADSVKDRFTISGDSAKHTMYLQMNSLKPEDTAVYYCGYNPGGWAVPSQYEYDSWGQGTQVTVSSAHHSEDPS

SEQ ID NO: 81 - protein, 124 aa, synthetic construct
QLQLVESGGGAAQTGGSLRLSCAASGGDSNINIMGWNRQVPGKQRELVAAITSDGNSNYGGSAKGRFTISRDNAKNTVYLQMNSLKPEDTAVYYCTVWTYSGKYEGQGTQVTVSSEPKTPKPQD

SEQ ID NO: 82 - protein, 116 aa, synthetic construct
ESGGGSVQTGGSLRLSCTASEYTYMNNCMGWFRQTPGKEREGIAAISSDGRRIEYDDSVKGRFVLSRDNDRNALILEMNALKSEDSGRYYCAAVRWGYPYSKSSYLGPGDPGHRLL

SEQ ID NO: 83 - protein, 410 aa, synthetic construct
ATGGCCCAGGTGCAGCTCGTGGAGTCAGGCGGAGGATTGGTGCAGGCTGGGGGCTCTCTGAGACTCTCCTGTGTAGCCTCTGGACGCGCCTTTCGTAGATATACCATGGGCTGGTTCCGCCAGGCTCCAGGGAAGGAGCGTGAGTTTGTAGCAACAATTAACTGGAGTGGTCGTAATACAGCGTATGCCGACTCCGTGAAGGGCCGATTCACCATCTCCAGAGACAGCCGCAAAAACACCGCGTATCTCCAAATGAACAGCCTGAAACCTGAAGATACGGCCGTTTATTATTGTGCACAATCGCGAGCGATTACAGGTGGCACAGTTCCCGCCGGTTATAACATCTGGGGCCAGGGGACCCAGGTCACCGTCTCCTCAGAACCCAAGACACCAAAACCACAAGCGGCCGC

SEQ ID NO: 84 - protein, 127 aa, synthetic construct
QVQLVESGGGLVHSGGSLRLSCAASGFTFSSEWMYWVRRDPLQWVSSINSPGSKTYYADSVRGRFTISRDNDKNMVYLQMNSLKPEDTGIYYCVRGVAQSVTGGEWYKVDLGDLEEWGQGTQVTVSS

SEQ ID NO: 85 - protein, 112 aa, synthetic construct
EVQLVESGGDQVQPGGSLRLSCVGSGFSFGTYTMMWFRHSPGKRLEWVSTINSDGSNPRYLNSVEDRFIISRDNAKNTLYLQMNNLKSEDTGLYYCTNGGTRGRGTQVTVSS